European Patent Application EP 4 140 497 A1, published March 1, 2023. Title: METHODS AND COMPOSITIONS FOR REJUVENATING SKELETAL MUSCLE STEM CELLS. Applicant: President and Fellows of Harvard College The Brigham and Women's Medical Center. Application 14782154.0. The sequence listing filed with the application follows.

SEQUENCE LISTING (4 sequences)

SEQ ID NO: 1 - protein, 346 aa, Homo sapiens
CPVCVWRQHSRELRLESIKSQILSKLRLKEAPNISREVVKQLLPKAPPLQQILDLHDFQGDALQPEDFLEEDEYHATTETVISMAQETDPAVQTDGSPLCCHFHFSPKVMFTKVLKAQLWVYLRPVPRPATVYLQILRLKPLTGEGTAGGGGGGRRHIRIRSLKIELHSRSGHWQSIDFKQVLHSWFRQPQSNWGIEINAFDPSGTDLAVTSLGPGAEGLHPFMELRVLENTKRSRRNLGLDCDEHSSESRCCRYPLTVDFEAFGWDWIIAPKRYKANYCSGQCEYMFMQKYPHTHLVQQANPRGSAGPCCTPTKMSPINMLYFNDKQQIIYGKIPGMVVDRCGCS

SEQ ID NO: 2 - protein, 337 aa, Homo sapiens
CNACTWRQNTKSSRIEAIKIQILSKLRLETAPNISKDVIRQLLPKAPPLRELIDQYDVQRDDSSDGSLEDDDYHATTETIITMPTESDFLMQVDGKPKCCFFKFSSKIQYNKVVKAQLWIYLRPVETPTTVFVQILRLIKPMKDGTRYTGIRSLKLDMNPGTGIWQSIDVKTVLQNWLKQPESNLGIEIKALDENGHDLAVTFPGPGEDGLNPFLEVKVTDTPKRSRRDFGLDCDEHSTESRCCRYPLTVDFEAFGWDWIIAPKRYKANYCSGECEFVFLQKYPHTHLVHQANPRGSAGPCCTPTKMSPINMLYFNGKEQIIYGKIPAMVVDRCGCS

SEQ ID NO: 3 - protein, 361 aa, Homo sapiens
RSSRPAPSVAPEPDGCPVCVWRQHSRELRLESIKSQILSKLRLKEAPNISREVVKQLLPKAPPLQQILDLHDFQGDALQPEDFLEEDEYHATTETVISMAQETDPAVQTDGSPLCCHFHFSPKVMFTKVLKAQLWVYLRPVPRPATVYLQILRLKPLTGEGTAGGGGGGRRHIRIRSLKIELHSRSGHWQSIDFKQVLHSWFRQPQSNWGIEINAFDPSGTDLAVTSLGPGAEGLHPFMELRVLENTKRSRRNLGLDCDEHSSESRCCRYPLTVDFEAFGWDWIIAPKRYKANYCSGQCEYMFMQKYPHTHLVQQANPRGSAGPCCTPTKMSPINMLYFNDKQQIIYGKIPGMVVDRCGCS

SEQ ID NO: 4 - protein, 361 aa, Mus musculus
RSSRPAPSAPPEPDGCPVCVWRQHSRELRLESIKSQILSKLRLKEAPNISREVVKQLLPKAPPLQQILDLHDFQGDALQPEDFLEEDEYHATTETVISMAQETDPAVQTDGSPLCCHFHFSPKVMFTKVLKAQLWVYLRPVPRPATVYLQILRLKPLTGEGTAGGGGGGRRHIRIRSLKIELHSRSGHWQSIDFKQVLHSWFRQPQSNWGIEINAFDPSGTDLAVTSLGPGAEGLHPFMELRVLENTKRSRRNLGLDCDEHSSESRCCRYPLTVDFEAFGWDWIIAPKRYKANYCSGQCEYMFMQKYPHTHLVQQANPRGSAGPCCTPTKMSPINMLYFNDKQQIIYGKIPGMVVDRCGCS